European Patent Specification EP 3 439 685 B1, published July 5, 2023. Title: Methods of Treating Cancer and Infectious Diseases Using Cell Based Therapies. Applicant: Emory University. The sequence listing filed with the application follows.

SEQUENCE LISTING (12 sequences)

SEQ ID NO: 1 - protein, 28 aa, Artificial
  Synthetic
KPRRPYTDNYTRLRKQMAVKKYLNSILN

SEQ ID NO: 2 - protein, 136 aa, Artificial
  Synthetic
MLLKLKEKASLTLAVGTLPFPSQFNFVPPGRMCRVAGWGRTGVLKPGSDTLQEVKLRLMDPQACSHFRDFDHNLQLCVGNPRKTKSAFKGDSGGPLLCAGVAQGIVSYGRSDAKPPAVFTRISHYRPWINQILQAN

SEQ ID NO: 3 - protein, 697 aa, Artificial
  Synthetic
DGICKSSDCIKSAARLIQNMDATTEPCTDFFKYACGGWLKRNVIPETSSRYGNFDILRDELEVVLKDVLQEPKTEDIVAVQKAKALYRSCINESAIDSRGGEPLLKLLPDIYGWPVATENWEQKYGASWTAEKAIAQLNSKYGKKVLINLFVGTDDKNSVNHVIHIDQPRLGLPSRDYYECTGIYKEACTAYVDFMISVARLIRQEERLPIDENQLALEMNKVMELEKEIANATAKPEDRNDPMLLYNKMTLAQIQNNFSLEINGKPFSWLNFTNEIMSTVNISITNEEDVVVYAPEYLTKLKPILTKYSARDLQNLMSWRFIMDLVSSLSRTYKESRNAFRKALYGTTSETATWRRCANYVNGNMENAVGRLYVEAAFAGESKHVVEDLIAQIREVFIQTLDDLTWMDAETKKRAEEKALAIKERIGYPDDIVSNDNKLNNEYLELNYKEDEYFENIIQNLKFSQSKQLKKLREKVDKDEWISGAAVVNAFYSSGRNQIVFPAGILQPPFFSAQQSNSLNYGGIGMVIGHEITHGFDDNGRNFNKDGDLVDWWTQQSASNFKEQSQCMVYQYGNFSWDLAGGQHLNGINTLGENIADNGGLGQAYRAYQNYIKKNGEEKLLPGLDLNHKQLFFLNFAQVWCGTYRPEYAVNSIKTDVESPGNFRIIGTLQNSAEFSEAFHCRKNSYMNPEKKCRVW

SEQ ID NO: 4 - protein, 29 aa, Artificial
  Synthetic
YFDAIFTNSYRKVLGQLSARKLLQDIMSR

SEQ ID NO: 5 - protein, 23 aa, Artificial
  Synthetic
FTDNYTRLRKQMAVKKYLNSILN

SEQ ID NO: 6 - protein, 28 aa, Artificial
  Synthetic
HSDAVFTDNYTRLRKQLAVKKYLNSILN

SEQ ID NO: 7 - protein, 6 aa, Artificial
  Synthetic
KPRRPY

SEQ ID NO: 8 - protein, 22 aa, Artificial
  Synthetic
TDNYTRLRKQMAVKKYLNSILN

SEQ ID NO: 9 - protein, 28 aa, Artificial
  Synthetic
  X (1)..(28): X is norleucine
KPRRPYTDNYTRLRKQXAVKKYLNSILN

SEQ ID NO: 10 - protein, 27 aa, Artificial
  Synthetic
HFDAVFTNSYRKVLKRLSARKLLQDIL

SEQ ID NO: 11 - protein, 32 aa, Artificial
  Synthetic
TDSYSRYRKQMAVKKYLAAVLGKRYKQRVKNK

SEQ ID NO: 12 - protein, 28 aa, Artificial
  Synthetic
HSDAVFTDNYTRLRKQMAVKKYLNSILN